European Patent Application EP 4 471 128 A1, published December 4, 2024. Title: 一种修饰的肿瘤浸润淋巴细胞及其用途. Applicant: 苏州沙砾生物科技有限公司. The sequence listing filed with the application follows.

SEQUENCE LISTING (68 sequences)

SEQ ID NO: 1 - RNA, 20 nt, synthetic construct
  modified_base 7: mod_base = OTHER; note = thymine
  modified_base 14: mod_base = OTHER; note = thymine
  misc_feature 1..20: note = gRNA knockout efficiency testing
  source 1..20: mol_type = other RNA
ggagaatgacgagtggaccc

SEQ ID NO: 2 - protein, 8 aa, synthetic construct
  REGION 1..8: note = OKT3 HCDR1
GYTFTRYT

SEQ ID NO: 3 - protein, 8 aa, synthetic construct
  REGION 1..8: note = OKT3 HCDR2
INPSRGYT

SEQ ID NO: 4 - protein, 12 aa, synthetic construct
  REGION 1..12: note = OKT3 HCDR3
ARYYDDHYSLDY

SEQ ID NO: 5 - protein, 5 aa, synthetic construct
  REGION 1..5: note = OKT3 LCDR1
SSVSY

SEQ ID NO: 6 - skipped

SEQ ID NO: 7 - protein, 9 aa, synthetic construct
  REGION 1..9: note = OKT3 LCDR3
QQWSSNPFT

SEQ ID NO: 8 - protein, 119 aa, synthetic construct
  REGION 1..119: note = OKT3 VH
QVQLVQSGGGVVQPGRSLRLSCKASGYTFTRYTMHWVRQAPGKGLEWIGYINPSRGYTNYNQKVKDRFTISRDNSKNTAFLQMDSLRPEDTGVYFCARYYDDHYSLDYWGQGTPVTVSS

SEQ ID NO: 9 - protein, 106 aa, synthetic construct [sequence omitted]

SEQ ID NO: 10 - protein, 222 aa, synthetic construct
  REGION 1..222: note = OKT3 heavy chain
QVQLVQSGGGVVQPGRSLRLSCKASGYTFTRYTMHWVRQAPGKGLEWIGYINPSRGYTNYNQKVKDRFTISRDNSKNTAFLQMDSLRPEDTGVYFCARYYDDHYSLDYWGQGTPVTVSSASTKGPSVFPLAPSSKSTSGGTAALGCLVKDYFPEPVTVSWNSGALTSGVHTFPAVLQSSGLYSLSSVVTVPSSSLGTQTYICNVNHKPSNTKVDKKVEPKSC

SEQ ID NO: 11 - protein, 213 aa, synthetic construct
  REGION 1..213: note = OKT3 light chain
DIQMTQSPSSLSASVGDRVTITCSASSSVSYMNWYQQTPGKAPKRWIYDTSKLASGVPSRFSGSGSGTDYTFTISSLQPEDIATYYCQQWSSNPFTFGQGTKLQITRTVAAPSVFIFPPSDEQLKSGTASVVCLLNNFYPREAKVQWKVDNALQSGNSQESVTEQDSKDSTYSLSSTLTLSKADYEKHKVYACEVTHQGLSSPVTKSFNRGEC

SEQ ID NO: 12 - protein, 5 aa, synthetic construct
  REGION 1..5: note = SP34 HCDR1
TYAMN

SEQ ID NO: 13 - protein, 19 aa, synthetic construct
  REGION 1..19: note = SP34 HCDR2
RIRSKYNNYATYYADSVKD

SEQ ID NO: 14 - protein, 14 aa, synthetic construct
  REGION 1..14: note = SP34 HCDR3
HGNFGNSYVSWFAY

SEQ ID NO: 15 - protein, 14 aa, synthetic construct
  REGION 1..14: note = SP34 LCDR1
RSSTGAVTTSNYAN

SEQ ID NO: 16 - protein, 7 aa, synthetic construct
  REGION 1..7: note = SP34 LCDR2
GTNKRAP

SEQ ID NO: 17 - protein, 9 aa, synthetic construct
  REGION 1..9: note = SP34 LCDR3
ALWYSNLWV

SEQ ID NO: 18 - protein, 125 aa, synthetic construct
  REGION 1..125: note = SP34 VH
EVQLVESGGGLVQPKGSLKLSCAASGFTFNTYAMNWVRQAPGKGLEWVARIRSKYNNYATYYADSVKDRFTISRDDSQSILYLQMNNLKTEDTAMYYCVRHGNFGNSYVSWFAYWGQGTLVTVSS

SEQ ID NO: 19 - protein, 109 aa, synthetic construct
  REGION 1..109: note = SP34 VL
QAVVTQESALTTSPGETVTLTCRSSTGAVTTSNYANWVQEKPDHLFTGLIGGTNKRAPGVPARFSGSLIGDKAALTITGAQTEDEAIYFCALWYSNLWVFGGGTKLTVL

SEQ ID NO: 20 - protein, 228 aa, synthetic construct
  REGION 1..228: note = SP34 heavy chain
EVQLVESGGGLVQPKGSLKLSCAASGFTFNTYAMNWVRQAPGKGLEWVARIRSKYNNYATYYADSVKDRFTISRDDSQSILYLQMNNLKTEDTAMYYCVRHGNFGNSYVSWFAYWGQGTLVTVSSASTKGPSVFPLAPSSKSTSGGTAALGCLVKDYFPEPVTVSWNSGALTSGVHTFPAVLQSSGLYSLSSVVTVPSSSLGTQTYICNVNHKPSNTKVDKKVEPKSC

SEQ ID NO: 21 - protein, 216 aa, synthetic construct
  REGION 1..216: note = SP34 light chain
QAVVTQESALTTSPGETVTLTCRSSTGAVTTSNYANWVQEKPDHLFTGLIGGTNKRAPGVPARFSGSLIGDKAALTITGAQTEDEAIYFCALWYSNLWVFGGGTKLTVLRTVAAPSVFIFPPSDEQLKSGTASVVCLLNNFYPREAKVQWKVDNALQSGNSQESVTEQDSKDSTYSLSSTLTLSKADYEKHKVYACEVTHQGLSSPVTKSFNRGEC

SEQ ID NO: 22 - protein, 8 aa, synthetic construct
  REGION 1..8: note = 15E8 HCDR1
GFSLTSYG

SEQ ID NO: 23 - protein, 7 aa, synthetic construct
  REGION 1..7: note = 15E8 HCDR2
IWAGGST

SEQ ID NO: 24 - protein, 17 aa, synthetic construct
  REGION 1..17: note = 15E8 HCDR3
ARDKRAPGKLYYGYPDY

SEQ ID NO: 25 - protein, 10 aa, synthetic construct
  REGION 1..10: note = 15E8 LCDR1
ESVEYYVTSL

SEQ ID NO: 26 - skipped

SEQ ID NO: 27 - protein, 9 aa, synthetic construct
  REGION 1..9: note = 15E8 LCDR3
QQTRKVPST

SEQ ID NO: 28 - protein, 123 aa, synthetic construct
  REGION 1..123: note = 15E8 VH 1
QVQLQESGPGLVKPSETLSLTCTVSGFSLTSYGVHWIRQPPGKGLEWLGVIWAGGSTNYNSSLKSRVTISKDTSKNQVFLKLSSVTADDTAVYYCARDKRAPGKLYYGYPDYWGQGTTLTVSS

SEQ ID NO: 29 - protein, 123 aa, synthetic construct
  REGION 1..123: note = 15E8 VH 2
QVQLQESGPGLVKPSETLSLTCTVSGFSLTSYGVHWIRQPPGKGLEWLGVIWAGGSTNYNSSLKSRVTISKDTSKNQVSLKLSSVTAADTAVYYCARDKRAPGKLYYGYPDYWGQGTTLTVSS

SEQ ID NO: 30 - protein, 111 aa, synthetic construct
  REGION 1..111: note = 15E8 VL
DIVMTQSPDSLAVSLGERATINCRASESVEYYVTSLMQWYQQKPGQPPKLLIYAASNVESGVPARFSGSGSGTDFTLTISPLQAEDVAVYYCQQTRKVPSTFGGGTKLEIK

SEQ ID NO: 31 - protein, 226 aa, synthetic construct
  REGION 1..226: note = 15E8 heavy chain 1
QVQLQESGPGLVKPSETLSLTCTVSGFSLTSYGVHWIRQPPGKGLEWLGVIWAGGSTNYNSSLKSRVTISKDTSKNQVFLKLSSVTADDTAVYYCARDKRAPGKLYYGYPDYWGQGTTLTVSSASTKGPSVFPLAPSSKSTSGGTAALGCLVKDYFPEPVTVSWNSGALTSGVHTFPAVLQSSGLYSLSSVVTVPSSSLGTQTYICNVNHKPSNTKVDKKVEPKSC

SEQ ID NO: 32 - protein, 226 aa, synthetic construct
  REGION 1..226: note = 15E8 light chain 2
QVQLQESGPGLVKPSETLSLTCTVSGFSLTSYGVHWIRQPPGKGLEWLGVIWAGGSTNYNSSLKSRVTISKDTSKNQVSLKLSSVTAADTAVYYCARDKRAPGKLYYGYPDYWGQGTTLTVSSASTKGPSVFPLAPSSKSTSGGTAALGCLVKDYFPEPVTVSWNSGALTSGVHTFPAVLQSSGLYSLSSVVTVPSSSLGTQTYICNVNHKPSNTKVDKKVEPKSC

SEQ ID NO: 33 - protein, 218 aa, synthetic construct
  REGION 1..218: note = 15E8 light chain
DIVMTQSPDSLAVSLGERATINCRASESVEYYVTSLMQWYQQKPGQPPKLLIYAASNVESGVPARFSGSGSGTDFTLTISPLQAEDVAVYYCQQTRKVPSTFGGGTKLEIKRTVAAPSVFIFPPSDEQLKSGTASVVCLLNNFYPREAKVQWKVDNALQSGNSQESVTEQDSKDSTYSLSSTLTLSKADYEKHKVYACEVTHQGLSSPVTKSFNRGEC

SEQ ID NO: 34 - DNA, 28 bp, synthetic construct
  source 1..28: mol_type = other DNA
gtaatcggcgtgcgaacggaatgtgcgg

SEQ ID NO: 35 - DNA, 28 bp, synthetic construct
  source 1..28: mol_type = other DNA
ctcaggggcccccagtagaatccgcagg

SEQ ID NO: 36 - RNA, 20 nt, synthetic construct
  modified_base 6: mod_base = OTHER; note = thymine
  modified_base 17: mod_base = OTHER; note = thymine
  modified_base 19: mod_base = OTHER; note = thymine
  misc_feature 1..20: note = SOCS1 gRNA 1
  source 1..20: mol_type = other RNA
cggcgtgcgaacggaatgtg

SEQ ID NO: 37 - RNA, 20 nt, synthetic construct
  modified_base 11: mod_base = OTHER; note = thymine
  modified_base 16: mod_base = OTHER; note = thymine
  misc_feature 1..20: note = SOCS1 gRNA 2
  source 1..20: mol_type = other RNA
gggcccccagtagaatccgc

SEQ ID NO: 38 - DNA, 28 bp, synthetic construct
  source 1..28: mol_type = other DNA
ggaagcttgtggcgctgaaaacgaacgg

SEQ ID NO: 39 - DNA, 28 bp, synthetic construct
  source 1..28: mol_type = other DNA
gcctttatgccatgagtgctcagagagg

SEQ ID NO: 40 - RNA, 20 nt, synthetic construct
  modified_base 2..3: mod_base = OTHER; note = thymine
  modified_base 5: mod_base = OTHER; note = thymine
  modified_base 11: mod_base = OTHER; note = thymine
  misc_feature 1..20: note = TNFAIP3 gRNA 1
  source 1..20: mol_type = other RNA
cttgtggcgctgaaaacgaa

SEQ ID NO: 41 - RNA, 20 nt, synthetic construct
  modified_base 1: mod_base = OTHER; note = thymine
  modified_base 3: mod_base = OTHER; note = thymine
  modified_base 8: mod_base = OTHER; note = thymine
  modified_base 12: mod_base = OTHER; note = thymine
  modified_base 15: mod_base = OTHER; note = thymine
  misc_feature 1..20: note = TNFAIP3 gRNA 2
  source 1..20: mol_type = other RNA
tatgccatgagtgctcagag

SEQ ID NO: 42 - DNA, 28 bp, synthetic construct
  source 1..28: mol_type = other DNA
tccaattccgcaaaatagagccccaagg

SEQ ID NO: 43 - DNA, 28 bp, synthetic construct
  source 1..28: mol_type = other DNA
caccttgcacagaactatcgtaccatgg

SEQ ID NO: 44 - DNA, 28 bp, synthetic construct
  source 1..28: mol_type = other DNA
cagcttgtgggatgtcgactcctagggg

SEQ ID NO: 45 - RNA, 20 nt, synthetic construct
  modified_base 1..2: mod_base = OTHER; note = thymine
  modified_base 11: mod_base = OTHER; note = thymine
  misc_feature 1..20: note = CB1 gRNA
  source 1..20: mol_type = other RNA
ttccgcaaaatagagcccca

SEQ ID NO: 46 - RNA, 20 nt, synthetic construct
  modified_base 1: mod_base = OTHER; note = thymine
  modified_base 11: mod_base = OTHER; note = thymine
  modified_base 13: mod_base = OTHER; note = thymine
  modified_base 16: mod_base = OTHER; note = thymine
  misc_feature 1..20: note = CB3 gRNA
  source 1..20: mol_type = other RNA
tgcacagaactatcgtacca

SEQ ID NO: 47 - RNA, 20 nt, synthetic construct
  modified_base 1: mod_base = OTHER; note = thymine
  modified_base 3: mod_base = OTHER; note = thymine
  modified_base 8: mod_base = OTHER; note = thymine
  modified_base 10: mod_base = OTHER; note = thymine
  modified_base 15: mod_base = OTHER; note = thymine
  modified_base 18: mod_base = OTHER; note = thymine
  misc_feature 1..20: note = CB2 gRNA
  source 1..20: mol_type = other RNA
tgtgggatgtcgactcctag

SEQ ID NO: 48 - DNA, 28 bp, synthetic construct
  source 1..28: mol_type = other DNA
gccctcagctccctctagtcccgcgggg

SEQ ID NO: 49 - DNA, 28 bp, synthetic construct
  source 1..28: mol_type = other DNA
ctggcctacgagtctgacgggatcgtgg

SEQ ID NO: 50 - DNA, 28 bp, synthetic construct
  source 1..28: mol_type = other DNA
ggtatggttcagaccagtactctcgagg

SEQ ID NO: 51 - RNA, 20 nt, synthetic construct
  modified_base 5: mod_base = OTHER; note = thymine
  modified_base 9: mod_base = OTHER; note = thymine
  modified_base 11: mod_base = OTHER; note = thymine
  modified_base 14: mod_base = OTHER; note = thymine
  misc_feature 1..20: note = ZC3 gRNA
  source 1..20: mol_type = other RNA
cagctccctctagtcccgcg

SEQ ID NO: 52 - RNA, 20 nt, synthetic construct
  modified_base 2: mod_base = OTHER; note = thymine
  modified_base 8: mod_base = OTHER; note = thymine
  modified_base 10: mod_base = OTHER; note = thymine
  modified_base 18: mod_base = OTHER; note = thymine
  misc_feature 1..20: note = ZC5 gRNA
  source 1..20: mol_type = other RNA
ctacgagtctgacgggatcg

SEQ ID NO: 53 - RNA, 20 nt, synthetic construct
  modified_base 3..4: mod_base = OTHER; note = thymine
  modified_base 13: mod_base = OTHER; note = thymine
  modified_base 16: mod_base = OTHER; note = thymine
  modified_base 18: mod_base = OTHER; note = thymine
  misc_feature 1..20: note = ZC7 gRNA
  source 1..20: mol_type = other RNA
ggttcagaccagtactctcg

SEQ ID NO: 54 - RNA, 19 nt, synthetic construct
  modified_base 7: mod_base = OTHER; note = thymine
  modified_base 13..14: mod_base = OTHER; note = thymine
  modified_base 16: mod_base = OTHER; note = thymine
  modified_base 19: mod_base = OTHER; note = thymine
  misc_feature 1..19: note = SC-4 gRNA
  source 1..19: mol_type = other RNA
gacgcctgcggattctact

SEQ ID NO: 55 - RNA, 20 nt, synthetic construct
  modified_base 1: mod_base = OTHER; note = thymine
  modified_base 3: mod_base = OTHER; note = thymine
  modified_base 6: mod_base = OTHER; note = thymine
  modified_base 19: mod_base = OTHER; note = thymine
  misc_feature 1..20: note = TP-N8 gRNA
  source 1..20: mol_type = other RNA
tgtcatagccgagaacaatg

SEQ ID NO: 56 - RNA, 20 nt, synthetic construct
  modified_base 1: mod_base = OTHER; note = thymine
  modified_base 6: mod_base = OTHER; note = thymine
  modified_base 9: mod_base = OTHER; note = thymine
  modified_base 11: mod_base = OTHER; note = thymine
  modified_base 19: mod_base = OTHER; note = thymine
  misc_feature 1..20: note = TP-N20 gRNA
  source 1..20: mol_type = other RNA
tcaactggtgtcgagaagtc

SEQ ID NO: 57 - RNA, 20 nt, synthetic construct
  modified_base 4: mod_base = OTHER; note = thymine
  modified_base 9: mod_base = OTHER; note = thymine
  modified_base 15: mod_base = OTHER; note = thymine
  modified_base 17: mod_base = OTHER; note = thymine
  misc_feature 1..20: note = ZC-11 gRNA
  source 1..20: mol_type = other RNA
agctggcctacgagtctgac

SEQ ID NO: 58 - RNA, 20 nt, synthetic construct
  modified_base 2: mod_base = OTHER; note = thymine
  modified_base 5: mod_base = OTHER; note = thymine
  modified_base 8: mod_base = OTHER; note = thymine
  modified_base 11: mod_base = OTHER; note = thymine
  modified_base 13: mod_base = OTHER; note = thymine
  misc_feature 1..20: note = ZC-13 gRNA
  source 1..20: mol_type = other RNA
gtcgtgatggtgtgaacacc

SEQ ID NO: 59 - DNA, 22 bp, synthetic construct
  misc_feature 1..22: note = SC-4 targeting sequence with PAM
  source 1..22: mol_type = other DNA
gacgcctgcggattctactggg

SEQ ID NO: 60 - DNA, 23 bp, synthetic construct
  misc_feature 1..23: note = TP-N8 targeting sequence with PAM
  source 1..23: mol_type = other DNA
tgtcatagccgagaacaatgggg

SEQ ID NO: 61 - DNA, 23 bp, synthetic construct
  misc_feature 1..23: note = TP-N20 targeting sequence with PAM
  source 1..23: mol_type = other DNA
tcaactggtgtcgagaagtccgg

SEQ ID NO: 62 - DNA, 23 bp, synthetic construct
  misc_feature 1..23: note = ZC-11 targeting sequence with PAM
  source 1..23: mol_type = other DNA
agctggcctacgagtctgacggg

SEQ ID NO: 63 - DNA, 23 bp, synthetic construct
  misc_feature 1..23: note = ZC-13 targeting sequence with PAM
  source 1..23: mol_type = other DNA
gtcgtgatggtgtgaacaccagg

SEQ ID NO: 64 - DNA, 25 bp, synthetic construct
  misc_feature 1..25: note = SC-4 25nt before PAM
  source 1..25: mol_type = other DNA
ctcctggacgcctgcggattctact

SEQ ID NO: 65 - DNA, 25 bp, synthetic construct
  misc_feature 1..25: note = TP-N8 25nt before PAM
  source 1..25: mol_type = other DNA
atggctgtcatagccgagaacaatg

SEQ ID NO: 66 - DNA, 25 bp, synthetic construct
  misc_feature 1..25: note = TP-N20 25nt before PAM
  source 1..25: mol_type = other DNA
gaaactcaactggtgtcgagaagtc

SEQ ID NO: 67 - DNA, 25 bp, synthetic construct
  misc_feature 1..25: note = ZC-11 25nt before PAM
  source 1..25: mol_type = other DNA
tgtgaagctggcctacgagtctgac

SEQ ID NO: 68 - DNA, 25 bp, synthetic construct
  misc_feature 1..25: note = ZC-13 25nt before PAM
  source 1..25: mol_type = other DNA
cacgcgtcgtgatggtgtgaacacc